European Patent Specification EP 3 110 948 B1, published April 9, 2025. Title: Variants of chymosin with improved milk-clotting properties. Applicant: Chr. Hansen A/S. The sequence listing filed with the application follows.

SEQUENCE LISTING (2 sequences)

SEQ ID NO: 1 - protein, 381 aa, Bos taurus
  SOURCE 1..381: /mol_type="protein" /organism="Bos taurus"
MRCLVVLLAVFALSQGAEITRIPLYKGKSLRKALKEHGLLEDFLQKQQYGISSKYSGFGEVASVPLTNYLDSQYFGKIYLGTPPQEFTVLFDTGSSDFWVPSIYCKSNACKNHQRFDPRKSSTFQNLGKPLSIHYGTGSMQGILGYDTVTVSNIVDIQQTVGLSTQEPGDVFTYAEFDGILGMAYPSLASEYSIPVFDNMMNRHLVAQDLFSVYMDRNGQESMLTLGAIDPSYYTGSLHWVPVTVQQYWQFTVDSVTISGVVVACEGGCQAILDTGTSKLVGPSSDILNIQQAIGATQNQYGEFDIDCDNLSYMPTVVFEINGKMYPLTPSAYTSQDQGFCTSGFQSENHSQKWILGDVFIREYYSVFDRANNLVGLAKAI

SEQ ID NO: 2 - protein, 381 aa, Camelus dromedarius
  SOURCE 1..381: /mol_type="protein" /organism="Camelus dromedarius"
MRCLVVLLAALALSQASGITRIPLHKGKTLRKALKERGLLEDFLQRQQYAVSSKYSSLGKVAREPLTSYLDSQYFGKIYIGTPPQEFTVVFDTGSSDLWVPSIYCKSNVCKNHHRFDPRKSSTFRNLGKPLSIHYGTGSMEGFLGYDTVTVSNIVDPNQTVGLSTEQPGEVFTYSEFDGILGLAYPSLASEYSVPVFDNMMDRHLVARDLFSVYMDRNGQGSMLTLGAIDPSYYTGSLHWVPVTLQQYWQFTVDSVTINGVAVACVGGCQAILDTGTSVLFGPSSDILKIQMAIGATENRYGEFDVNCGNLRSMPTVVFEINGRDYPLSPSAYTSKDQGFCTSGFQGDNNSELWILGDVFIREYYSVFDRANNRVGLAKAI